European Patent Specification EP 3 655 029 B1, published March 18, 2026. Title: Immunogenic Composition. Applicant: GlaxoSmithKline Biologicals SA. The sequence listing filed with the application follows.

SEQUENCE LISTING (66 sequences)

SEQ ID NO: 1 - protein, 5 aa, Artificial
  consensus sequence
  MISC_FEATURE (1)..(1): Xaa="Asp" or "Glu"
  MISC_FEATURE (2)..(2): Xaa="Ala" or "Arg" or "Asn" or "Asp" or "Cys" or "Gln" or "Glu" or "Gly" or "His" or "Ile" or "Leu" or "Lys" or "Met" or "Phe" or "Ser" or "Thr" or "Trp" or "Tyr" or "Val"
  MISC_FEATURE (4)..(4): Xaa="Ala" or "Arg" or "Asn" or "Asp" or "Cys" or "Gln" or "Glu" or "Gly" or "His" or "Ile" or "Leu" or "Lys" or "Met" or "Phe" or "Ser" or "Thr" or "Trp" or "Tyr" or "Val"
  MISC_FEATURE (5)..(5): Xaa="Ser" or "Thr"
XXNXX

SEQ ID NO: 2 - protein, 5 aa, Artificial
  consensus sequence
DQNAT

SEQ ID NO: 3 - protein, 7 aa, Artificial
  consensus sequence
  MISC_FEATURE (2)..(2): Xaa="Asp" or "Glu"
  MISC_FEATURE (3)..(3): Xaa="Ala" or "Arg" or "Asn" or "Asp" or "Cys" or "Gln" or "Glu" or "Gly" or "His" or "Ile" or "Leu" or "Lys" or "Met" or "Phe" or "Ser" or "Thr" or "Trp" or "Tyr" or "Val"
  MISC_FEATURE (5)..(5): Xaa="Ala" or "Arg" or "Asn" or "Asp" or "Cys" or "Gln" or "Glu" or "Gly" or "His" or "Ile" or "Leu" or "Lys" or "Met" or "Phe" or "Ser" or "Thr" or "Trp" or "Tyr" or "Val"
  MISC_FEATURE (6)..(6): Xaa="Ser" or "Thr"
KXXNXXK

SEQ ID NO: 4 - protein, 7 aa, Artificial
  consensus sequence
KDQNATK

SEQ ID NO: 5 - protein, 481 aa, Streptococcus pneumoniae
MSRRFKKSGSQKVKRSVNIVLLTIYLLLVCFLLFLIFKYNILAFRYLNLVVTALVLLVALVGLLLIIYKKAEKFTIFLLVFSILVSSVSLFAVQQFVGLTNRLNATSNYSEYSISVAVLADSDIENVTQLTSVTAPTGTDNENIQKLLADIKSSQNTDLTVNQSSSYLAAYKSLIAGETKAIVLNSVFENIIESEYPDYASKIKKIYTKGFTKKVEAPKTSKNQSFNIYVSGIDTYGPISSVSRSDVNILMTVNRDTKKILLTTTPRDAYVPIADGGNNQKDKLTHAGIYGVDSSIHTLENLYGVDINYYVRLNFTSFLKLIDLLGGIDVYNDQEFTAHTNGKYYPAGNVHLDSEQALGFVRERYSLADGDRDRGRNQQKVIVAILQKLTSTEALKNYSTIINSLQDSIQTNMPLETMINLVNAQLESGGNYKVNSQDLKGTGRTDLPSYAMPDSNLYVMEIDDSSLAVVKAAIQDVMEGR

SEQ ID NO: 6 - protein, 243 aa, Streptococcus pneumoniae
MIDIHSHIVFDVDDGPKSREESKALLTESYRQGVRTIVSTSHRRKGMFETPEEKIAENFLQVREIAKEVADDLVIAYGAEIYYTLDALEKLEKKEIPTLNDSRYALIEFSMNTPYRDIHSALSKILMLGITPVIAHIERYDALENNGKRVRELIDMGCYTQINSYHVSKPKFFGEKYKFMKKRARYFLERDLVHVVASDMHNLDSRPPYMQQAYDIIAKKYGAKKAKELFVDNPRKIIMDQLI

SEQ ID NO: 7 - protein, 230 aa, Streptococcus pneumoniae
MKEQNTLEIDVLQLFRALWKRKLVILLVAIITSSVAFTYSTFVIKPEFTSTTRIYVVNRNQGEKSGLTNQDLQAGTYLVKDYREIILSQDVLEEVVSDLKLDLTPKGLANKIKVTVPVDTRIVSVSVNDRVPEEASRIANSLREVAAQKIISITRVSDVTTLEEARPAISPSSPNIKRNILIGFLAGVIGTSVIVLLLELLDTRVKRPEDIEDTLQMTLLGVVPNLNKLK

SEQ ID NO: 8 - protein, 227 aa, Streptococcus pneumoniae
MPTLEIAQKKLEFIKKAEEYYNALCTNIQLSGDKLKVISVTSVSPGEGKTTTSVNIAWSFARAGYKTLLIDGDTRNSVISGFFKSREKITGLTEFLSGTADLSHGLCDTNIENLFVVQSGSVSPNPTALLQSKNFNDMIETLRKYFDYIIVDTAPIGIVIDAAIITQKCDASILVTATGEANKRDVQKAKQQLKQTGKLFLGVVLNKLDISVDKYGVYGFYGNYGKK

SEQ ID NO: 9 - protein, 455 aa, Streptococcus pneumoniae
MDEKGLKIFMAVLQSIIVILLVYFLSFVRETELERSSMVILYLLHFFVFYVSSYGNNFFKRGYLVEFNSTIRYIFFFAIAISVLNFFIAERFSISRRGMVYFLTLEGISLYLLNFLVKKYWKHVFFNLKNSKKILLLTVTKNMEKVLDKLLESDELSWKLVAVSVLNKSDFQHDKIPVIEKEKIIEFATHEVVDEVFVNLPGESYDIGEIISRFETMGIDVTVNLKAFDKNLGRNKQIHEMVGLNVVTFSTNFYKTSHVISKRILDICGATIGLILFAIASLVLVPLIRKDGGPAIFAQTRIGKNGRHFTFYKFRSMRIDAEAIKEQLMDQNTMQGGMFKIDNDPRVTKIGRFIRKTSLDELPQFWNVFIGDMSLVGTRPPTVDEYDQYTPEQKRRLSFKPGITGLWQVSGRSKITDFDDVVKLDVSYIDNWTIWKDIEILLKTVKVVFMRDGAK

SEQ ID NO: 10 - protein, 392 aa, Streptococcus pneumoniae
MKKSVYIIGSKGIPAKYGGFETFVEKLTAFQQDKAIQYYVACMRENSAKSGTTEDVFEHNGAICYNVDVPNIGPARAIVYDIAAINRAIEIAKENKDEDPIFYILACRIGPFIHGIKKKIQAIGGTLLVNPDGHEWLRAKWSTPVRRYWKISEGLMVKHADLLVCDSKNIEQYIQEDYKQFQPKTTYIAYGTDTTRSILKSSDEKVRSWFKEKNVSENEYYLVVGRFVPENNYESMILGFLASNSKKDFVLITNVEQNKFYNQLLAKTGFDKDPRVKFVGTVYNQELLKYIRENAFAYFHGHEVGGTNPSLLEALASTKLNLLLDVGFNREVAEDGADYWEKDNLHKVIEASEQKTQEEINEKNILSTKQVTERFSWDLIVNEYEKLFTRKN

SEQ ID NO: 11 - protein, 468 aa, Streptococcus pneumoniae
MRYGIMRISFSKKTMLCGLLYIGLILSVVTIPTIVTFLYSLLFIGIVTVLNYNSILASDEDANSFFVALPIILSSFQNVYLGFGADRLNSVTLQVLLSISIAIITITVFLGIILNRFKSKEFSWLVLSILVIIIQSVILLIFFPTTLPAYLSSMRNILAPLLIFYFSIYGFKNINLQKFYKYMFIIILVVLIFGFIEYIYGNSLWTRLNIKKLWALKGLAIENRVVPGNWHSSELIGGKQLRRMVSTFADPVNLGSYLFAAFMLAWYKNKKLLQVLLLASFVLSVSKAAFLSMLVYIIIYTWVVDKNKILSIFGIIISTVLGLYFYNFSQVSSYGSINAHIDGFFSALSTPLHYPFGMGVGSVGVLASKLGSQTALSSEVLETGIGMIIAQLGFVGVIIYLIFFVKLSVIGKNINNKRDKILWFTLIYSFLANAFFNEVALSPNSCTLYFLILGLLYNKNKIRSTEFS

SEQ ID NO: 12 - protein, 323 aa, Streptococcus pneumoniae
MEKLVSIILPVYNVEQYIKNCLESIQQQTYPNLEVIIVNDGSTDKSVEYCEQICKIDSRFSITHKENGGLSDARNVGIDKAKGDYLIFVDSDDFVSQDMVSYLVSCMENNEADIAICDPVHYYSDRQNNDLNIFSPASSVKVYETTEALCEMFYQKSFLVSAWAKIFKRELFDDIRFPVGKLFEDSAIMYLLLEKCETIAYSDAKLYAYVHRDNSITTKKFSDRDLDILEITNTIINHYGDNLRVYTAAVSYKVSACFRILLNSPSEEKYKKVQKECLSYILQNWRNILFNNNVRLKNKLALISITIFNPFVKLIYSKVNRWE

SEQ ID NO: 13 - protein, 410 aa, Streptococcus pneumoniae
MNKYEERYQENLSKNDFYKLINKSYLSDKELQVQQVKAGIVLPPKAFETKLSNKLGLQKSLHGKGGVVDSNGNYIELSAQKAVGMRNRVYGPYKINYDNLPIRNEKVIYLNYFIKQWGHFLLDVVGRLWYPLLQDNDTKLVYTCYAGTETKIEGNYLEFLKLLGIDQSRLIMINCPTQFSEVIIPESSILPGGYYTKEYKQLFSSVVENIKLDKYDVNAKMIYCSRSKLGIAKSKEFGEDGIEGIFKQNGYTSVYMETMSLEEQIKTLLSAKTIVLTSGSLAHNLLFVNKDIDVFILNKTYRVNLHQFLINEISDATVRFVDIYRSPLPILYGYGPFLMDLTKPLANFLDDNEFVYEKGTVLSKKDYFKYYLKWLWSYRFFLFRLNGIKEGNSEFEKSFKIIRRYYKTGR

SEQ ID NO: 14 - protein, 461 aa, Streptococcus pneumoniae
MSKYKELAKNTGIFALANFSSKILIFLLVPIYTRVLTTTEYGFYDLVYTTIQLFVPILTLNISEAVMRFLMKDGVSKKSVFSIAVLDIFIGSIAFALLLLVNNLFSLSDLISQYSIYIFVIFVFYTLNNFLIQFSKGIDKIGVTAISGVISTAVMLAMNVILLVVFDWGLLGFFIANVCGYVIPCIYIVSRLRLWELFEIKIDKKLQWEMVYYALPLVLNILSWWVNNTSDRYIVTAIVGIQASAIISVAYKIPQILSTISAIFIQSWQISAIKIQEDKSGTTFVSNMLLYYNALLLIIASGIILFVKPISNILFGISFYSAWELVPFLIISSLFNAISGCIGAIMGAKMDTHNIAKSALVGMIANIILNIVLTFLMGPQGITISTLIASFLIFYMRKDSVKEINSETYRAIYLSWILLVVEACLLIYMDFIIGALIAMVINLFLLKDVIKPLYLKIFKRN

SEQ ID NO: 15 - protein, 382 aa, Streptococcus pneumoniae
MIVLQYFKILARFVFMFLISAVLLPFKIKPNKIVFINFNGKGYGDNPKSICEYLRTTYPDLDLVWLARDNEGFPDGVRVVKYGTFQAFYEQASSKVWVYNVRAFARILKKRGQIYIQTWHGASSFKLIEKQADLPINYVLEAKYDARVTDIMISDSRKQTEEFQKYFWYSGEIFEVGMPRNDALFHYKEDYDKLNNIRKELSIHSDDYVILYAPTFRDDGDASYLDINFERLLQCVEHGIKKKCKFLIRLHPNHSHLCNNISFNKNIINATFYSDMQELTLLADVLVTDYSSSIFDFMLLNKPYVRYVNDLEKYAELRGVSDTYYELPDSIIKTAEELYDLLPKKIENFDYDSIKKYRNEILCPIFNGTASENVGRRIIQEL

SEQ ID NO: 16 - protein, 342 aa, Streptococcus pneumoniae
MKNNDLKIGSGAIHQISATLSQNSISGKILYCADPVVDDLYGSIVRSQIEEIGRVKEESCNYNTIAYAMNIAERAIATDIDCIVGMGGGRVLDVCKYASFISKRPYLSIPTTAANDGIASPVAVLKRQDDRPKSLGAAIPSMTLIDIDVIASGPIQNIKAGIGDTISNYTALKDWELAVERGKDEMHGFAYLMSQNSLDALMKTKYNSITPDFIEVLVNSLVLSGIAMDFAGSSRPVSGSEHLFSHALDYYGSTRNLHGIQVALGTVAVLKLIENSVDTVVDYLQRFEVHINPKLLGIDEELFIYCMQHATKMRSNRYTYLHEVDLSTDRLKQIYKELISEL

SEQ ID NO: 17 - protein, 234 aa, Streptococcus pneumoniae
MKALILAAGLGTRLAPITNEVPKSLVPVNGKPILMKQIENLYQNNITDITIIAGYKSSVLTDAVTEKYPEINIIDNVDFKTTNNMYSAYLGKAAMGDSDFLMMNADVFYDASVIKSLLLHKAPNAIVTDLGIYIEESMKVVEKNGRLVEISKQISPEETLGASIDVYKFSYEAGARFFEKCKEFIEDKRELQMWSEVALNAILSEVEFVACPLEGRWLEIDNHEDLVAAEKLFA

SEQ ID NO: 18 - protein, 277 aa, Streptococcus pneumoniae
MKLTNRVDYFGADISELQNKKLFLFDMDGTIYEEDRLFEGTLELLDYIHNIGGEYIFITNNSSKSVVDYVEKVNRLGIKAERDNFFTSAQATIVYIKENYPKSKVYCQGTKSLIKELSDAGIDVTEQVSADIDVVLVGFDTELTSDKIRNTCEILSTKDVPFIATNPDIRCPVSFGFIPDCGSICDMISKSVDRKPVYIGKPEPTMVDIVRKKLNYSLFETVVIGDRLYTDIMTGINAGVTSVCVLTGEATVNDIQQDSIKPTYTFKNVKEMWKGIV

SEQ ID NO: 19 - protein, 289 aa, Streptococcus pneumoniae
MKGIILAGGSGTRLYPLTRAASKQLMPVYDKPMIYYPLSTLMLAGIRDILIISTPQDLPRFKELLQDGSEFGIKLSYAEQPSPDGLAQAFIIGEEFIGDDSVALILGDNIYHGPGLSTMLQKAAKKEKGATVFGYHVKDPERFGVVEFDENMNAISIEEKPEYPRSNYAVTGLYFYDNDVVEIAKSIKPSPRGELEITDVNKAYLDRGDLSVELMGRGFAWLDTGTHESLLEASQYIETVQRMQNVQVANLEEIAYRRGYISREDVLALAQSLKKNEYGQYLLRLIGEA

SEQ ID NO: 20 - protein, 197 aa, Streptococcus pneumoniae
MTDNFFGKTLAARKVEAIPGMLEFDIPVHGDNRGWFKENFQKEKMLPLGFPESFFAEGKLQNNVSFSRKNVLRGLHAEPWDKYISVADGGKVLGSWVDLREGETFGNTYQTVIDASKGIFVPRGVANGFQVLSDTVSYSYLVNDYWALELKPKYAFVNYADPSLGIEWENIAEAEVSEADKNHPLLKDVKPLKKEDL

SEQ ID NO: 21 - protein, 349 aa, Streptococcus pneumoniae
MTEYKNIIVTGGAGFIGSNFVHYVYENFPDVHVTVLDKLTYAGNRANIEEILGNRVELVVGDIADAELVDKLAAQADAIVHYAAESHNDNSLNDPSPFIHTNFIGTYTLLEAARKYDIRFHHVSTDEVYGDLPLREDLPGHGEGPGEKFTAETKYNPSSPYSSTKAASDLIVKAWVRSFGVKATISNCSNNYGPYQHIEKFIPRQITNILSGIKPKLYGEGKNVRDWIHTNDHSSGVWTILTKGQIGETYLIGADGEKNNKEVLELILKEMGQAVDAYDHVTDRAGHDLRYAIDASKLRDELGWKPEFTNFEAGLKATIKWYTDNQEWWKAEKEAVEANYAKTQEIITV

SEQ ID NO: 22 - protein, 283 aa, Streptococcus pneumoniae
MILITGANGQLGTELRYLLDERNEEYVAVDVAEMDITDAEMVEKVFEEVKPTLVYHCAAYTAVDAAEDEGRELDFAINVTGTKNVAKASEKHGATLVYISTDYVFDGKKPVGQEWEVDDRPDPQTEYGRTKRMGEELVEKHVSNFYIIRTAWVFGNYGKNFVFTMQNLAKTHKTLTVVNDQYGRPTWTRTLAEFMTYLAENRKEFGYYHLSNDATEDTTWYDFAVEILKGTDVEVKPVDSSQFPAKAKRPLNSTMSLAKAKATGFVIPTWQDALQEFYKQEVR

SEQ ID NO: 23 - protein, 484 aa, Streptococcus pneumoniae
MLIMSRRFKKSGSQKVKRSVNIVLLTIYLLLVCFLLFLIFKYNILAFRYFNLVVTALVLLVALVGLLLIIYKKAEKFTIFLLVFSILVSSVSLFAVQQFVGLTNRLNATSNYSEYSISVAVLADSDIENVTQLTSVTAPTGTDNENIQKLLADIKSSQNIDLTVNQSSSYLAAYKSLIAGETKAIVLNSVFENIIESEYPDYASKIKKIYTKGFTKKVEAPKTSKNQSFNIYVSGIDTYGPISSVSRSDVNILMTVNRDTKKILLTTTPRDAYVPIADGGNNQKDKLTHAGIYGVDSSIHTLENLYGVDIHYYVRLNFTSFLKLIDLLGGVDVYNDQDFTSLHGKFHFPVGNVHLDSEQALGFVRERYSLADGDHDRGRNQQKVIAAILQKLTSSEALKNYSMIIDSLQDSIQTNMPLETMINLVNAQLESGGTYKVNSQDLKGRGRTDLPSYAMPDSNLYMMEINDSSLASVKTAIQDVLEGR

SEQ ID NO: 24 - protein, 259 aa, Streptococcus pneumoniae
MHLSKLLFRMCWRADEMIDIHSHIVFDVDDGPKSREESKALLTEAYRQGVRTIVSTSHRRKGMFETPEEKIAENFLQVREIAKEVASDLVIAYGAEIYYTPDVLGKLEKNRIPTLNNSRYALIEFSMNTPYRDIHSALIKILMLGITPVIAHIERYDALENNEKRVRELINMGCYTQVNSSHVLKSKLFGEPYKFMKKRAQYFLERDLVHVIASDMHNVDSRPPHMAEAYDLVSQKYGETKAQDLFIDNPRKIVMDQLI

SEQ ID NO: 25 - protein, 230 aa, Streptococcus pneumoniae
MKEQNTIEIDVFQLLKTLWKHKLIILLVALVTGAGAFAYSIFIVKPEYTSTTRIYVVNRNQENKPGLTNQDLQAGTYLVKDYHEIILSQDVLEKVATNLKLDIPVKTLTSKVQVTVPADTRIVSISVKDKQPEEASRIANSIREVAAEKIIAVTRVSDVTTLEEARPATTPSSPNVRRNTLVGFLGAAAVTVITVLLIELFDTRVKRPEEVEDVLQMPLLGVVPDFNKMK

SEQ ID NO: 26 - protein, 229 aa, Streptococcus pneumoniae
MPTLEISQAKLELAKKTEEYYNALCTNPQLSGDDLKVFSISSVKAGEGKTTTSTNIAWAFAHAGYKTLLIDADMRNSVMSGVFKSRERITGLTEFLSGTTDLSQGLCDTNVENLFVIQAGSVSPNPIALLQSKNFSTMLGTLRKYFDYIVVDTAPIGIVIDAAIIMQKCDASILVTKAGETKRRELQKAKEQLEQTGKSCLGVVLNKFDTSVDKYGFYGSYGSYRKQKK

SEQ ID NO: 27 - protein, 453 aa, Streptococcus pneumoniae
MNEKLAKSSVAIVQSFLVILLTYLLSAVRETEIVSTTAIVLYILHYFVFYISDYGRNFFKRRYLIELVQTLKYILFFALAISISNFFLEDRFSISRRGMIYFLLLHVFLVYMLNLFIKWYWKRAYPNFKGSKKVFLLTATSHVEKVLDRLIESDDVVGELVAVSVLDKPDFQHDDLKVVAEGEIVNFATREVVDEVFINLPSEKYNIGELVSQFETMGIDVTVNLNAFDWARNKQICEMAGLNVVTFSTTFYKTSHVIAKRVIDIIGSLVGLILCGLVSIVLVPLIRKDGGSAIFAQTRIGKNGRHFTFYKFRSMCVDAEDKKRELMEQNTMQGGMFKVDDDPRITKIGHFIRKTSLDELPQFYNVLKGDMSLVGTRPPTVDEYEHYTPEQKRRLSFKPGITGLWQVSGRSEIKNFDEVVKLDVVYIDGWTIWKDIEILLKTVKVVLMKDGAK

SEQ ID NO: 28 - protein, 407 aa, Streptococcus pneumoniae
MERNSLLLFQTIRRKMKKSVYIIGSKGIPAKYGGFETFVEKLTEYQKDGNIQYYVACMRENSAKSGFTADTFEYNDAICYNIDVPNIGPARAIAYDIAAVNKAIEIAKKNKDEAPIFYILACRIGPFIARLKKKIQAIGGTLFVNPDGHEWLRAKWSLPVRKYWKFSEQLMVKYADLLVCDSKNIEKYIQNDYKQYQPKTTYIAYGTDTSPSILKSEDLKIRSWYQEKGLSENGYYLVVGRFVPENNYETMIREFIKSKSKKDFVLITNVEQNKFYDQLLQETGFDKDPRVKFVGTVYDQELLKYIRENAFAYFHGHEVGGTNPSLLEALASTKLNLLLDVGFNREVGEDGAIYWRKDNLHKVIEESEQKTIEEIKEIDILSTEQVEKRFTWDFIVNEYENLFLLGK

SEQ ID NO: 29 - protein, 395 aa, Streptococcus pneumoniae
MTIKINYMFFVCLSFFGIVLSSSQVIVNLGLSSIVQYIAYFLLLLCIFFTLIKNSPDVIANRIAYFSIISFLFIIGINLQNLPFSTKIYLSFSMLIISSLSTLPIKLINNINDFRRISYFLLNGILLSTFLGWLFNISLVTVAVEGIGFAYGFNGGLTHKNFYAITILVSYILLFISRKHGTKYQVDSLVLWFDLFLLLVSNTRTIYIILVVFWIVVHSGFIKYIKKNHRPVIITTWLVISLLSIIFFFKHIINNSESYTHRVLGIVNFFKYYESSKFHLFFGDAELAFGDMTKGYTHNIRSVLGWDGTVEMPLLSVMIKNGYVGLIGYGVVLFKFISSVLSMEDRRVKNIGLSILIPLLLSAMVENYIVNISFVFMPVCFCILCSIKNIEFKNN

SEQ ID NO: 30 - protein, 322 aa, Streptococcus pneumoniae
MKKVSIILPVYNVEQYIKKCLESIQQQTYPNLEVIIVNDGATDKSVEYCEQICKIDSRFSVTHKENGGLSDARNVGIDKAKGDYLIFVDSDDFVSQDMVSYLVSSMENNEADIAICDPAHYYSDRQNNDLNIFYPASSVKVYEKTEALCEMFYQKSFLVSAWAKIYKKELFDDIRFPVGKLFEDSAVMYLLFEKCEKIVYSNAKLYAYVHRDNSITTKKFSDKDLDILDISNTILDHYSGNFRVYKAAVSYKVSACFRILLNSSSEKKYNQIQKDCMTYILRNWRNMLFDKNVRLKNKLALISITLFNPFVKFIYSKVNRWE

SEQ ID NO: 31 - protein, 412 aa, Streptococcus pneumoniae
MNKYEERYQEDLSKNDFEKLINRRYLSDKELQVEYVKKGTVLPPKVFEMKLSNKLGLQKALHGKGGVVDSKGNYVELSEQKAVGMRNRVYGSYKFNHKNLAIRNEKVIYLNYFINQWGHFLLDVVGRLWYPLLKDTDTKLDYTCYAGTETKLEGNYLEFLELLGIDKSRLILINRPTQFSEIIIPESSILPGEYYTKEYKMLFNSLVANVKLDNNLESKKIYCSRARLDLAKGKEFGENGIEKVFLKNGYTPVYMETMSLKEQIRTLLSATTIVLTSGSLAHNLLFINNKINVFILNKTYRVNLHQFLINKISEASVSFVDIYRSPLPILYGYGPFLMDITKPLVNFFEDSGFTYDSGTILDKTDYFKFYLKWLWSYKFFLFRLNHIKEGNSEFEKSFKIIRRYYKMGRQYE

SEQ ID NO: 32 - protein, 462 aa, Streptococcus pneumoniae
MSKYKELAKNTGTFALANFSSKILIFLLVPIYTKVLTTTEYGFYDLVYTTIQLLVPILTLNISEAVMRFLMKEDVSKKSVFSIAILDIFLGSIIFCLLLLVNQIFSLSELISQYSIYIMAIFAFYTLNNFLIQYSKGIDKIGVTAISGVISAAVMLSMNILLLVVLNWGLLGFFIANICGYVIPCVYIIVKLKLWDLFELKIDRSLQWEMIYYTLPLILNTLSWWVNNTSDRYIITVIIGIQASAIISVAYKIPQIFSTISAIFIQSWQISAIKIQEEKEGNTFISKMLLYYNALLLIIASGIILFVKPISNILFGASFYSAWTLVPFLIISSLFNAISGYIGAIMGAKMDTKNIAKSALVGMIANVFLNIVLTFLMGLQGITISTMIASFLIFYMRKDSVEEIAPETYRAIYLSWFLLVVEASLLVYIDFIIGATLVTLINLFLLKDTLKPLCLKLLKGFK

SEQ ID NO: 33 - protein, 384 aa, Streptococcus pneumoniae
MKMNILQYIKILARTIFMLLISTVLLPVRLKNNKILFINFNGKGYGDNPKSICEYLRTTYPDLDLVWLARDNEGFPDGVRVVKYGTFQAFYEQASSKVWVYNVRAFARILKKRGQIYIQTWHGASSFKLIEKQADLPINYVLEAKYDARVTDIMISDSRKQTEEFQKYFWYSGEIFEVGMPRNDALFHYKEDYDKLNNIRKELSIHSDDYVILYAPTFRDDGDASYLDINFERLLQCVEHGIKKKCKFLIRLHPNHSHLCNNISFNKNIINATFYSDMQELTLLADVLVTDYSSSIFDFMLLNKPYVRYVNDLEKYAELRGVSDTYYELPDSIIKTAEELYDLLPKKIENFDYDSIKKYRNEILCPIFNGTASENVGRRIIQEL

SEQ ID NO: 34 - protein, 342 aa, Streptococcus pneumoniae; identical to SEQ ID NO: 16

SEQ ID NO: 35 - protein, 234 aa, Streptococcus pneumoniae; identical to SEQ ID NO: 17

SEQ ID NO: 36 - protein, 283 aa, Streptococcus pneumoniae
MNRIRRMKLTNRVDYFGADISELQNKKLFLFDMDGTIYEEDRLFEGTLELLDYIHNIGGEYIFITNNSSKSVVDYVEKVNRLGIKAERDNFFTSAQATIVYIKENYPKSKVYCQGTKSLIKELSDAGIDVTEQVSADIDVVLVGFDTELTSDKIRNTCEILSTKDVPFIATNPDIRCPVSFGFIPDCGSICDMISKSVDRKPVYIGKPEPTMVDIVRKKLNYSLFETVVIGDRLYTDIMTGINAGVTSVCVLTGEATVNDIQQDSIKPTYTFKNVKEMWKGIV

SEQ ID NO: 37 - protein, 289 aa, Streptococcus pneumoniae
MKGIILAGGSGTRLYPLTRAASKQLMPVYDKPMIYYPLSTLMLAGIRDILIISTPQDLPRFKELLQDGSEFGIKLSYAEQPSPDGLAQAFIIGEEFIGDDSVALILGDNIYHGPGLSTMLQKAAKKEKGATVFGYHVKDPERFGVVEFDENMNAISIEEKPEYPRSNYAVTGLYFYDNDVVEIAKSIKPSPRGELEITDVNKAYLDRGDLSVELMGRGFAWLDTGTHESLLEASQYIETVQRMQNVQVANLEEIAYRMGYISREDVLALAQPLKKNEYGQYLLRLIGEA

SEQ ID NO: 38 - protein, 197 aa, Streptococcus pneumoniae; identical to SEQ ID NO: 20

SEQ ID NO: 39 - protein, 349 aa, Streptococcus pneumoniae (
MTEYKNIIVTGGAGFIGSNFVHYVYENFPGVHVTVLDKLTYAGNRANIEEILGNRVELVVGDIADAELVDKLAAQADAIVHYAAESHNDNSLNDPSPFIHTNFIGTYTLLEAARKYDIRFHHVSTDEVYGDLPLREDLPGHGEGPGEKFTAETKYNPSSPYSSTKAASDLIVKAWVRSFGVKATISNCSNNYGPYQHIEKFIPRQITNILSGIKPKLYGEGKNVRDWIHTNDHSSGVWTILTKGQIGETYLIGADGEKNNKEVLELILKEMGQATDAYDHVTDRAGHDLRYAIDASKLRDELGWKPEFTNFEAGLKATIKWYTDNQEWWKAEKEAVEANYAKTQEIITV

SEQ ID NO: 40 - protein, 283 aa, Streptococcus pneumoniae
MILITGANGQLGTELRYLLDERNEEYVAVDVAEMDITNEEMVEKVFEEVKPTLVYHCAAYTAVDAAEDEGKELNFAINVTGTKNVAKASEKHGATLVYISTDYVFDGKKPVGQEWEVDDRPDPQTEYGRTKRMGEELVEKHVSNFYIIRTAWVFGNYGKNFVFTMQNLAKTHKTLTVVNDQYGRPTWTRTLAEFMTYLAENRKEFGYYHLSNDATEDTTWYDFAVEILKDTDVEVKPVDSSQFPAKAKRPLNSTMSLAKAKATGFVIPTWQDALQEFYKQEVR

SEQ ID NO: 41 - protein, 481 aa, Streptococcus pneumoniae
MSRRFKKSRSQKVKRSVNIVLLTIYLLLVCFLLFLIFKYNILAFRYLNLVVTALVLLVALVGLLLIIYKKAEKFTIFLLVFSILVSSVSLFAVQQFVGLTNRLNATSNYSEYSISVAVLADSDIENVTQLTSVTAPTGTDNENIQKLLADIKSSQNTDLTVDQSSSYLAAYKSLIAGETKAIVLNSVFENIIESEYPDYASKIKKIYTKGFTKKVEAPKTSKNQSFNIYVSGIDTYGPISSVSRSDVNILMTVNRDTKKILLTTTPRDAYVPIADGGNNQKDKLTHAGIYGVDSSIHTLENLYGVDINYYVRLNFTSFLKMIDLLGGVDVHNDQEFSALHGKFHFPVGNVHLDSEQALGFVRERYSLADGDRDRGRNQQKVIVAILQKLTSTEALKNYSTIIDSLQDSIQTNMPLETMINLVNAQLESGGNYKVNSQDLKGTGRTDLPSYAMPDSNLYVMEIDDSSLAVVKAAIQDVMEGR

SEQ ID NO: 42 - protein, 243 aa, Streptococcus pneumoniae
MIDIHSHIVFDVDDGPKSREESKALLTESYRQGVRTIVSTSHRRKGMFETPEEKIAENFLQVREIAKEVADDLVIAYGAEIYYTLDALEKLEKKEIPTLNDSRYALIEFSMNTPYRDIHSALSKILMLGITPVIAHIERYDALENNEKRVRELIDMGCYTQVNSSHVLKPKLFGERYKFMKKRAQYFLEQDLVHVIASDMHNLDGRPPHMAEAYDLVTQKYGEAKAQELFIDNPRKIVMDQLI

SEQ ID NO: 43 - protein, 231 aa, Streptococcus pneumoniae
MMKEQNTIEIDVFQLFKTLWKRKLMILIVALVTGTGAFAYSTFIVKPEYTSTTRIYVVNRNQGDKPGLTNQDLQAGTYLVKDYREIILSQDALEKVATNLKLDMPAKTLASKVQVAVPADTRIVSISVKDKQPEEASRIANSLREVAAEKIVAVTRVSDVTTLEEARPATTPSSPNVRRNSLFGFLGGAVVTVIAVLLIELLDTRVKRPEDVEDVLKIPLLGLVPDFDKIK

SEQ ID NO: 44 - protein, 229 aa, Streptococcus pneumoniae
MPTLEISQAKLDSVKKAEEYYNALCTNLQLSGDGLKVFSITSVKIGEGKSTTSANIAWAFARAGYKTLLIDGDIRNSVMLGVFKARNKITGLTEFLSGTTDLSQGLCDTNIENLFVIQAGSVSPNPTALLQSKNFTTMLETLRKYFDYIIVDTAPVGVVIDAAIITRNCDASILVTEAGEINRRDIQKAKEQLEHTGKPFLGIVLNKFDTSVDKYGSYGNYGNYGKNKK

SEQ ID NO: 45 - protein, 455 aa, Streptococcus pneumoniae
MNEKILRSSLAIIQSFLVILLTYLLSAVRETEIVSTTAIALCILHYFVFYISDYGQDFFKRRYLIELVQTLKYILFFALAIGISNFFLEDRFSISRRGMIYFLTLHALLVYVLNLFIKWYWKRAYPNFKGSKKILLLTATSRVEKVLDRLIESNEVVGKLVAVSVLDKPDFQHDCLKVVAEGGIVNFATHEVVDEVFINLPSEKYNIGELVSQFETMGIDVIVNLNAFDRSLARNKQIREMAGLNVVTFSTTFYKTSHVIAKRIIDIVGALVGLILCGLVSIVLVPLIRKDGGSAIFAQTRIGKNGRQFTFYKFRSMCVDAEAKKRELMEQNTMQGGMFKVDDDPRITKIGCFIRKTSLDELPQFYNVLKGDMSLVGTRPPTVDEYEHYTPEQKRRLSFKPGITGLWQVSGRSEIKNFDEVVKLDVAYIDGWTIWKDIEILLKTVKVVFMRDGAK

SEQ ID NO: 46 - protein, 392 aa, Streptococcus pneumoniae
MKKSVYIIGSKGIPAKYGGFETFVEKLTAFQQDKAIQYYVACMRENSAKSGTTEDVFEHNGAICYNVDVPNFGPARAIAYDIAAINRAIEIAKENKDEDPIFYILACRIGPFIHGIKKKIQEIGGTLLVNPDGHEWLRAKWSAPVRRYWKISEGLMVKHADLLVCDSKNIEKYIQEDYKQYQPKTTYIAYGTDTTRSVLKSSDEKVRSWFKEKNVSENEYYLVVGRFVPENNYESMIRGFLASNSKKDFVLITNVEQNKFYNQLLAKTGFDKDPRVKFVGTVYEQELLKYIRENAFAYFHGHEVGGTNPSLLEALASTKLNLLLDVGFNREVAEDGAIYWKKDNLHEIIETSEQKTQKEIDEKDILSIKQVTERFSWELIVNEYEKLFLCEK

SEQ ID NO: 47 - protein, 397 aa, Streptococcus pneumoniae
MTIKINNLFFVCLSFFGIVLSSSQVIVNLGLSSIIQYISYFMLMLCVFLTLIKNTLNVFANRIIYFLIISFLFIIGINLQNLPLSRKIYLSFSMLIISSLSTLPIKLINNLSDLRRISYYLLHSIFLSVFLGLVFKISLVTVAVEGIGFSYGFNGGLTHKNFYAITILVSYILLYVSRKYDAKHQIDSFVLWLDLFLLLISNTRTVYIILVVFWIIINRNFINNIKKEHRLVVTATTIVISLLALTFFFKHIINNSESYSHRVLGVVNFFKYYESDRFHLFFGDAELAFGNTTKGYGHNIRSVLGWDGTVEMPLLSVMIKNGYVGLVGYIIVLFKFISSIISVKNSTKKNIGLSIFIPLLLSATVENYIVNISFVFMPVCFCILCSIKNIKLVNNRK

SEQ ID NO: 48 - protein, 323 aa, Streptococcus pneumoniae
MEKLVSIILPVYNVEQYIKNCLESIQQQTYSNLEVIIVNDGSTDKSVEYCEQICKIDSRFSITHKENGGLSDARNVGIDKSKGDYLIFVDSDDFVSQDMVSYLVSCMENNEADIAICDPVHYYSDRQNNDLNIFSPASNVKVYETTEALCEMFYQKSFLVSAWAKIFKRELFDDIRFPVGKLFEDSAIMYLLFEKCETIAYSDAELYAYVHRDNSITTKKFSDRDLDILEITNTIINHYGDNLRVYTAAVSYKVSACFRILLNSPSGEKYKKVQKECLSYILQNWRNILFNNNVRLKNKLALISITIFNPFVKFIYSKVNRWE

SEQ ID NO: 49 - protein, 410 aa, Streptococcus pneumoniae; identical to SEQ ID NO: 13

SEQ ID NO: 50 - protein, 461 aa, Streptococcus pneumoniae
MSKYKELAKNTGIFALANFSSKILIFLLVPIYTRVLTTTEYGFYDLVYTTIQLFVPILTLNISEAVMRFLMKDGVSKKSVFSIAVLDIFIGSIAFALLLLVNNLFSLSDLISQYSIYIFVIFVFYTLNNFLIQFSKGIDKIGVTAISGVISTAVMLAMNVILLVVFDWGLLGFFIANVCGYVIPCIYIVSRLRLWELFEIKIDKKLQWEMVYYALPLVLNILSWWVNNTSDRYIVTAIVGIQASAIISVAYKIPQILSTISAIFIQSWQISAIKIQEDKSDTTFVSNMLLYYNALLLIIASGIILFVKPISNILFGISFYSAWELVPFLIISSLFNAISGCIGAIMGAKMDTHNIAKSALVGMIANIILNIVLTFLMGPQGITISTLIASFLIFYMRKDSVKEINSETYRAIYLSWILLVVEACLLIYMDFIIGALIAMVINLFLLKDVIKPLYLKIFKRN

SEQ ID NO: 51 - protein, 382 aa, Streptococcus pneumoniae; identical to SEQ ID NO: 15

SEQ ID NO: 52 - protein, 342 aa, Streptococcus pneumoniae; identical to SEQ ID NO: 16

SEQ ID NO: 53 - protein, 234 aa, Streptococcus pneumoniae; identical to SEQ ID NO: 17

SEQ ID NO: 54 - protein, 277 aa, Streptococcus pneumoniae; identical to SEQ ID NO: 18

SEQ ID NO: 55 - protein, 289 aa, Streptococcus pneumoniae; identical to SEQ ID NO: 19

SEQ ID NO: 56 - protein, 197 aa, Streptococcus pneumoniae; identical to SEQ ID NO: 20

SEQ ID NO: 57 - protein, 349 aa, Streptococcus pneumoniae; identical to SEQ ID NO: 21

SEQ ID NO: 58 - protein, 283 aa, Streptococcus pneumoniae; identical to SEQ ID NO: 22

SEQ ID NO: 59 - protein, 358 aa, E. coli
MEENNMKTVAVVGTVGVPACYGGFESLVQNLIDYQSDGIQYQIFCSSKKYDKKFKNYKNAELIYLPINANGVSSIIYDIMCLIICLFKRPDVVLILGVSGCLFLPIYKLFSKSKIIVNIDGLEWRRNKWGTFAKKFLKISEAISIRIADIIISDNQAIADYVENKYKKKSVVIAYGGDHATNLSTPIDNDQKKEGYYLGLCRIEPENNIEMILNAFINTDKKIKFMGNWDNSEYGRQLKKYYSNYPNITLLEPNYNIEELYKLRKNCLAYIHGHSAGGTNPSLVEAMHFNIPIFAFDCDFNRYTTNNLAHYFNDSEQLSLLAESLSFGNLKCRVLDLKNYAEDMYNWRHIAAMYESIY

SEQ ID NO: 60 - protein, 360 aa, E. coli
MTEQFSEKKIDVVGIVGLPACYGGFESLVQNLVDYQSQNIKYNVYCSRKKYKNTPKKYKRADLKYIPFDANGSSSILYDIYSLFLSLFNKVDVVLILGVSGCVFLPIYRFFSSSKVIVNIDGLEWKRAKWKGIAKWYLKISEKIAVKYSDVVVADNEAIAKYVLKKYGLEAKIIAYGGDHSLVKKPISVIKEDYFFTVCRIEPENNIRMILEAFKNTTHSLKIVGNWDSSLYGRRLKEEFGNYNNIEIIDPIYDSDILFNFRSLCRGYIHGHSAGGTNPSLVEAMHFQIPIIAFDCDFNRFTTDNYAFYFKNKNELSFIVNDILNGNQNEQAEICAKKMKEIATKKYTWDTIAKMYEELY

SEQ ID NO: 61 - protein, 351 aa, Cronobacter sakazakii
MKRIAVVGTVGIPACYGGFESLVENLTKYKGAGYQYYIFCSSKNYPEKSDSHNDAQLIYVPLKANGIQSILYDIVSLWKCLFLKVDTILILGVSGCIFLPVFRLLSNAKIITNIDGLEWKREKWNYPIKKFLKFSELLAVKYSHAIVTDNRAITDYVKKEYNVSSFTIAYGGDHAVRPSNNNNNIKSSYALGLCRIEPENNVELILKAFTLSEDKLKFVGNWNASSYGRMLKKNYSNYSNIELIEPIYDIDKLYILRSGCDKYIHGHSAGGTNPSLVEMMHFGVPIFAFDCEFNRHSTDNKAFYFKDAQHLADLVKMKDNTELEKNSCNMKVLAQENYTWQKITASYESLY

SEQ ID NO: 62 - protein, 664 aa, Campylobacter jejuni
IISNDGYAFAEGARDMIAGFHQPNDLSYYGSSLSTLTYWLYKITPFSFESIILYMSTFLSSLVVIPIILLANEYKRPLMGFVAALLASIANSYYNRTMSGYYDTDMLVIVLPMFILFFMVRMILKKDFFSLIALPLFIGIYLWWYPSSYTLNVALIGLFLIYTLIFHRKEKIFYIAVILSSLTLSNIAWFYQSTIIVILFALFALEQKRLNFVIIGILASVTLIFLILSGGVDPILYQLKFYIFRSDESANLTQGFMYFNVNQTIQEVENVDLSEFMRRISGSEIVFLFSLFGFVWLLRKHKSMIMALPILVLGFLALKGGLRFTIYSVPVMALGFGFLLSEFKAILVKKYSQLTSNVCIVFATILTLAPVFIHIYNYKAPTVFSQNEASLLNQLKNIANREDYVVTWWDYGYPVRYYSDVKTLVDGGKHLGKDNFFPSFALSKDEQAAANMARLSVEYTEKSFYAPQNDILKTDILQAMMKDYNQSNVDLFLASLSKPDFKIDTPKTRDIYLYMPARMSLIFSTVASFSFINLDTGVLDKPFTFSTAYPLDVKNGEIYLSNGVVLSDDFRSFKIGDNVVSVNSIVEINSIKQGEYKITPIDDKAQFYIFYLKDSAIPYAQFILMDKTMFNSAYVQMFFLGNYDKNLFDLVINSRDAKVFKLKI

SEQ ID NO: 63 - protein, 257 aa, E. coli
MMVFGKLYLSSLGYIFGSWEMVLGPFGYFLTLFAVWAAINAFNMVDGIDGLLGGLSCVSFAAIGMILWFDGQTSLAIWCFAMIAAILPYIMLNLGILGRRYKVFMGDAGSTLIGFTVIWILLETTQGKTHPISPVTALWIIAIPLMDMVAIMYRRLRKGMSPFSPDRQHIHHLIMRAGFTSRQAFVLITLAAALLASIGVLAEYSHFVPEWVMLVLFLLAFFLYGYCIKRAWKVARFIKRVKRRLRRNRGGSPNLTK

SEQ ID NO: 64 - protein, 207 aa, E. coli
MSTIIMDLCSYTRLGLTGYLLSRGVKKREINDIETVDDLAIACDSQRPSVVFINEDCFIHDASNSQRIKLIINQHPNTLFIVFMAIANVHFDEYLLVRKNLLISSKSIKPESLDDILGDILKKETTITSFLNMPTLSLSRTESSMLRMWMAGQGTIQISDQMNIKAKTVSSHKGNIKRKIKTHNKQVIYHVVRLTDNVTNGIFVNMR

SEQ ID NO: 65 - protein, 713 aa, Campylobacter jejuni
MLKKEYLKNPYLVLFAMIILAYVFSVFCRFYWVWWASEFNEYFFNNQLMIISNDGYAFAEGARDMIAGFHQPNDLSYYGSSLSALTYWLYKITPFSFESIILYMSTFLSSLVVIPTILLANEYKRPLMGFAAALLASIANSYYNRTMSGYYDTDMLVIVLPMFILFFMVRMILKKDFFSLIALPLFIGIYLWWYPSSYTLNVALIGLFLIYTLIFHRKEKIFYIAVILSSLTLSNIAWFYQSAIIVILFALFALEQKRLNFMIIGILGSATLIFLILSGGVDPILYQLKFYIFRSDESANLTQGFMYFNVNQTIQEVENVDLSEFMRRISGSEIVFLFSLFGFVWLLRKHKSMIMALPILVLGFLALKGGLRFTIYSVPVMALGFGFLLSEFKAIMVKKYSQLTSNVCIVFATILTLAPVFIHIYNYKAPTVFSQNEASLLNQLKNIANREDYVVTWWDYGYPVRYYSDVKTLVDGGKHLGKDNFFPSFALSKDEQAAANMARLSVEYTEKSFYAPQNDILKTDILQAMMKDYNQSNVDLFLASLSKPDFKIDTPKTRDIYLYMPARMSLIFSTVASFSFINLDTGVLDKPFTFSTAYPLDVKNGEIYLSNGVVLSDDFRSFKIGDNVVSVNSIVEINSIKQGEYKITPIDDKAQFYIFYLKDSAIPYAQFILMDKTMFNSAYVQMFFLGNYDKNLFDLVINSRDAKVFKLKI

SEQ ID NO: 66 - protein, 378 aa, Salmonella typhimurium
MPSLNVKQEKNQSFAGYSLPPANSHEIDLFSLIEVLWQAKRRILATVFAFACVGLLLSFLLPQKWTSQAIVTPAESVQWQGLERTLTALRVLDMEVSVDRGSVFNLFIKKFSSPSLLEEYLRSSPYVMDQLKGAQIDEQDLHRAIVLLSEKMKAVDSNVGKKNETSLFTSWTLSFTAPTREEAQKVLAGYIQYISDIVVKETLENIRNQLEIKTRYEQEKLAMDRVRLKNQLDANIQRLHYSLEIANAAGIKRPVYSNGQAVKDDPDFSISLGADGISRKLEIEKGVTDVAEIDGDLRNRQYHVEQLAAMNVSDVKFTPFKYQLSPSLPVKKDGPGKAIIIILAALIGGMMACGGVLLRHAMVSRKMENALAIDERLV